European Patent Application EP 4 450 631 A1, published October 23, 2024. Title: 氧化还原酶及其突变体在生物合成圆柚酮中的应用. Applicant: 华南理工大学. Application CN 202111517500.9, filed December 13, 2021. The sequence listing filed with the application follows.

SEQUENCE LISTING (22 sequences)

SEQ ID NO: 1 - DNA, 795 bp, (Artificial Sequence)
  misc_feature 1..795: note = NRRL
  source 1..795: mol_type = other DNA
atgactttaaacacccaaaagaaaacagcattagttacaggagcagctcaaggtattgggaaatccattgcaattcaattagctaaagatggttaccaagttgcaattacagatttaccatttcaaaaggcgaaagcattagaaacagttaaagagattgaaaaatttggagcagaatcactatttattccatgtgattcatctaagaaacaagaaatctttgatgcggttgatgaaacctataaaaaatttggtgggtttgataccattgttaataatgctggtattgcaactatagcacctattgtggaaacgacagaagaggaaatcaataaaatcttgagtattaatgttaatggtgttgtgtttgggattcaagcagctgcaaagaagtttgaagaattgggaaatcaaccaggtaaaatcatcaatgcagcttcgattgtttcatatgaagcatttgaaatgttgggtatttatagtgcgactaagtttgcagttcgtgggttaactcaagttgctgctaaagaattggcttcaagaaagattactgttaattgttactgcccagggattgtattaacaccaatgtgggatcaaattgatgctaaaatgggtgaatattcaggcgcagctaaaggagagaccgttaagaagtttattgacaagattgcacttggaagaggatctgaacctcaagacgttgccaacttggttagtttcatggctagtgaaaaggctgattatattacgggacaagctatggttgttgatggtggaataatgtatcattaa

SEQ ID NO: 2 - protein, 264 aa, (Artificial Sequence)
  REGION 1..264: note = NRRL
MTLNTQKKTALVTGAAQGIGKSIAIQLAKDGYQVAITDLPFQKAKALETVKEIEKFGAESLFIPCDSSKKQEIFDAVDETYKKFGGFDTIVNNAGIATIAPIVETTEEEINKILSINVNGVVFGIQAAAKKFEELGNQPGKIINAASIVSYEAFEMLGIYSATKFAVRGLTQVAAKELASRKITVNCYCPGIVLTPMWDQIDAKMGEYSGAAKGETVKKFIDKIALGRGSEPQDVANLVSFMASEKADYITGQAMVVDGGIMYH

SEQ ID NO: 3 - DNA, 795 bp, (Artificial Sequence)
  misc_feature 1..795: note = NRRL
  source 1..795: mol_type = other DNA
atgactttgaacactcaaaagaaaactgctttggttactggtgctgctcaaggtattggtaaatctattgctattcaattggctaaggatggctaccaagttgctattactgatttgccattccaaaaggctaaggctttggaaactgttaaggaaattgaaaagttcggtgctgaatctttgttcattccatgtgattcttctaagaagcaagaaattttcgatgctgttgatgaaacttataagaaattcggtggtttcgatactattgttaataatgccggtatcgctactatcgctccaattgttgaaactacagaagaagaaattaataagattttatctattaatgttaacggtgttgttttcggtattcaagccgctgctaagaagttcgaagaattgggtaaccaaccaggtaaaattattaatgctgcttctatcgtttcctacgaagcttttgaaatgttgggtatctactccgctactaagtttgctgttagaggtttaactcaagttgctgctaaggaattggcctccagaaaaattactgttaactgttactgtccaggtattgttttgactccaatgtgggatcaaattgacgctaagatgggtgaatattccggtgctgctaagggtgaaactgttaagaaattcattgataagattgctttgggtagaggttctgaaccacaagatgttgctaacttagtttcctttatggcttctgaaaaggctgattatattactggtcaagctatggttgttgacggtggtattatgtaccattaa

SEQ ID NO: 4 - protein, 264 aa, (Artificial Sequence)
  REGION 1..264: note = K69T-G136R
MTLNTQKKTALVTGAAQGIGKSIAIQLAKDGYQVAITDLPFQKAKALETVKEIEKFGAESLFIPCDSSTKQEIFDAVDETYKKFGGFDTIVNNAGIATIAPIVETTEEEINKILSINVNGVVFGIQAAAKKFEELRNQPGKIINAASIVSYEAFEMLGIYSATKFAVRGLTQVAAKELASRKITVNCYCPGIVLTPMWDQIDAKMGEYSGAAKGETVKKFIDKIALGRGSEPQDVANLVSFMASEKADYITGQAMVVDGGIMYH

SEQ ID NO: 5 - DNA, 50 bp, (Artificial Sequence)
  misc_feature 1..50: note = NRRL-F
  source 1..50: mol_type = other DNA
agtttcgaataaacacacataaacaaacaaaatgactttaaacacccaaa

SEQ ID NO: 6 - DNA, 50 bp, (Artificial Sequence)
  misc_feature 1..50: note = NRRL-R
  source 1..50: mol_type = other DNA
gaccaaacctctggcgaagaagtccaaagctttaatgatacattattcca

SEQ ID NO: 7 - DNA, 50 bp, (Artificial Sequence)
  misc_feature 1..50: note = TDH3-F
  source 1..50: mol_type = other DNA
tgaccatgattacgaattctttaccgtcgacacagtttattcctggcatc

SEQ ID NO: 8 - DNA, 50 bp, (Artificial Sequence)
  misc_feature 1..50: note = TDH3-R
  source 1..50: mol_type = other DNA
gaccaaacctctggcgaagaagtccaaagcttttgtttgtttatgtgtgt

SEQ ID NO: 9 - DNA, 48 bp, (Artificial Sequence)
  misc_feature 1..48: note = ADH1-F
  source 1..48: mol_type = other DNA
gaataaacacacataaacaaacaaaagctttggacttcttcgccagag

SEQ ID NO: 10 - DNA, 50 bp, (Artificial Sequence)
  misc_feature 1..50: note = ADH1-R
  source 1..50: mol_type = other DNA
ttgcatgcctgcaggtcgactctagaggatccatagggtaggggaatttc

SEQ ID NO: 11 - DNA, 24 bp, (Artificial Sequence)
  misc_feature 1..24: note = YEp352-F1
  source 1..24: mol_type = other DNA
gatcctctagagtcgacctgcagg

SEQ ID NO: 12 - DNA, 26 bp, (Artificial Sequence)
  misc_feature 1..26: note = YEp352-R1
  source 1..26: mol_type = other DNA
gtcgacggtaaagaattcgtaatcat

SEQ ID NO: 13 - DNA, 19 bp, (Artificial Sequence)
  misc_feature 1..19: note = YEp352-F2
  source 1..19: mol_type = other DNA
agctttggacttcttcgcc

SEQ ID NO: 14 - DNA, 20 bp, (Artificial Sequence)
  misc_feature 1..20: note = YEp352-R2
  source 1..20: mol_type = other DNA
tttgtttgtttatgtgtgtt

SEQ ID NO: 15 - DNA, 26 bp, (Artificial Sequence)
  misc_feature 1..26: note = YEp352-F3
  source 1..26: mol_type = other DNA
gtgaccgtctccgggagctgcatgtg

SEQ ID NO: 16 - DNA, 26 bp, (Artificial Sequence)
  misc_feature 1..26: note = YEp352-R3
  source 1..26: mol_type = other DNA
ccggagacggtcacagcttgtctgta

SEQ ID NO: 17 - DNA, 26 bp, (Artificial Sequence)
  misc_feature 1..26: note = NRRL(cp)K69T-F
  source 1..26: mol_type = other DNA
cttctacgaagcaagaaattttcgat

SEQ ID NO: 18 - DNA, 26 bp, (Artificial Sequence)
  misc_feature 1..26: note = NRRL(cp)K69T-R
  source 1..26: mol_type = other DNA
cttgcttcgtagaagaatcacatgga

SEQ ID NO: 19 - DNA, 26 bp, (Artificial Sequence)
  misc_feature 1..26: note = NRRL(cp)G136R-F
  source 1..26: mol_type = other DNA
aattgcgtaaccaaccaggtaaaatt

SEQ ID NO: 20 - DNA, 25 bp, (Artificial Sequence)
  misc_feature 1..25: note = NRRL(cp)G136R-R
  source 1..25: mol_type = other DNA
tggttacgcaattcttcgaacttct

SEQ ID NO: 21 - DNA, 26 bp, (Artificial Sequence)
  misc_feature 1..26: note = NRRL(cp)G136A-F
  source 1..26: mol_type = other DNA
aattggctaaccaaccaggtaaaatt

SEQ ID NO: 22 - DNA, 25 bp, (Artificial Sequence)
  misc_feature 1..25: note = NRRL(cp)G136A-R
  source 1..25: mol_type = other DNA
tggttagccaattcttcgaacttct